European Patent Application EP 4 592 389 A2, published July 30, 2025. Title: ANALYSIS OF TARGET MOLECULES WITHIN A SAMPLE VIA HYBRIDIZATION CHAIN REACTION. Applicant: California Institute of Technology. Application EP. The sequence listing filed with the application follows.

SEQUENCE LISTING (4 sequences)

SEQ ID NO: 1 - DNA, 78 bp, synthetic construct
  misc_feature 1..78: note = Synthetic; Hairpin H1 including toehold for auxiliary strand nucleation
  source 1..78: mol_type = other DNA
cgggttaaagttgagtggagatatagaggcagggacaaagtctaatccgtccctgcctctatatctccactctatcat

SEQ ID NO: 2 - DNA, 72 bp, synthetic construct
  misc_feature 1..72: note = Synthetic; Hairpin H2
  source 1..72: mol_type = other DNA
gtccctgcctctatatctccactcaactttaacccggagtggagatatagaggcagggacggattagacttt

SEQ ID NO: 3 - DNA, 36 bp, synthetic construct
  misc_feature 1..36: note = Synthetic; Initiator I1
  source 1..36: mol_type = other DNA
gtccctgcctctatatctccactcaactttaacccg

SEQ ID NO: 4 - DNA, 42 bp, synthetic construct
  misc_feature 1..42: note = Synthetic; Auxiliary strand
  source 1..42: mol_type = other DNA
atgatagagtggagatatagaggcagggacggattagacttt